European Patent Specification EP 4 114 975 B1, published April 29, 2026. Title: Fascin-2 (FSCN2) Variants And Uses Thereof. Applicant: Regeneron Pharmaceuticals, Inc. PRAVEEN, Kavita COPPOLA, Giovanni GURSKI, Lauren FERRIERA, Manuel Allen Revez DRUMMOND, Meghan BARAS, Aris ABECASIS, Goncalo. The sequence listing filed with the application follows.

SEQUENCE LISTING (22 sequences)

SEQ ID NO: 1 - DNA, 8735 bp, Homo sapien
cagggggttcgtgacgccggctgggtctgggggctgtgggccagccgagccgacccgggcttctgggggaccgcgggggccgtgagcactcagagggcgcatcccaggcccctccggggacccggccagcctgaagatgccgacgaacggcctgcaccaggtgctgaagatccagtttggcctcgtcaacgacactgaccgctacctgacagctgagagcttcggcttcaaggtcaatgcctcggcacccagcctcaagaggaagcagacctgggtgctggaacccgacccaggacaaggcacggctgtgctgctccgcagcagccacctgggccgctacctgtcggcagaagaggacgggcgcgtggcctgtgaggcagagcagccgggccgtgactgccgcttcctggtcctgccgcagccagatgggcgctgggtgctgcggtccgagccgcacggccgcttcttcggaggcaccgaggaccagctgtcctgcttcgccacagccgtttccccggccgagctgtggaccgtgcacctggccatccacccgcaggcccacctgctgagcgtgagccggcggcgctacgtgcacctgtgcccgcgggaggacgagatggccgcagacggagacaagccctggggcgtggacgccctcctcaccctcatcttccggagccgacggtactgcctcaagtcctgtgacagccgctacctgcgcagcgacggccgtctggtctgggagcctgagccccgtgcctgctacacgctggagttcaaggcgggcaagctggccttcaaggactgcgacggccactacctggcacccgtggggcccgcaggcaccctcaaggccggccgaaacacgcgacctggcaaggatgagctctttgatctggaggagagtcacccacaggtggtgctggtggctgccaaccaccgctacgtctctgtgcggcaaggtagggagggcacaggtggcgacctcctgaggggtgctgggacccccctgcttcagggaggaggccgtgggggtctcacggggagtggtatcgtgtctgtgcgttcacatgtctgttctgggctgggggtccatgtgggacatgtgtggccactcagggtgtaggtgggtgggcctcgggccatgcccaggcgacccccactgaggggtggtggcttcagggtcagaggcaagggttcctggcctttctcagcatagctggagaatgtctcagccaagccctgggcagctgcggagtctgagactggagaggtgtgggccaggcgatgggcagtgcccagcaggggcaggaggcccacagcctggcctggtgccatgaggggcatgtgggcaggaggctgtggggggtccatatctccccttctttttctccaccccattttctggacttcatttatttatttattttttgagacagagtctcgctctgtcacccaggctggagcgcagtggcgtgatctcggctcactgcaagcgccgcctcacgggttcacgccattctcctgcctcagcctcccgagtagctgggactacaggcgcccgccaccacgcccggctaattttttgtattttttagaagagacggggtttcactgtgttagccaggatggtcttgatctcctgaccttgtgatctgtccacctcggcctcccaaagtgctgggattacaggcgtgagccaccgtgcccggctgcattttctggactttaaaggaaattggggaggagcccagggtagggcagggagctggggatcgggcggggatagcaccaccacgtgcctgaccagtggagcctcgtgtcctcaggagtgggggggcttaaggtcagctccagtgatggaggacacggtgggcaggcagctttacccggggcctgggctcctggtggggaggcacctccctgccccagtggggcgtggcctggctctccccagttcccaggtcaccagttgcctgtctgtgtgactccctccaccgcctatggggtgaaccccagcagttcctccttccccacaagctgagctctgagggaaaagccctggcccgggcagtcactacccacctgggctcctggctccatgcaccccagagtggctcggaggtggtctgaaaaggcgaggtggggagagccgggtgcatggagctcctcctcccaactcaggtccttccagaccagcatcagctgggcaaggagagctcccctgtctcctggcagctcccaggtgcccaccaagcccccaccctgacggatgtccaggccccctgggtacactgacactctggggccagatggcagaggccccaccctgtgcatggagaggggagcccagccatggctatggggtcctgcacctgcagttggcatcctcgggcctgtcccagcagtgacagggtcccaggagtgagaattcaactgtggatgcacggccatggcccttccttcctatcacagcccacagtccagctgtaatgcctgctggcctgggcccaggccgggcatgtggcaatccttaggtggttaaagggggtaagtgggacagtggcagtgagaatgcttcctccatggaagccaaagacactagacctttaggcatttgtatatggacagcttggaaagcagactcaaagtggcagtcatggccgtggccgtggcattgtggtgtgatgtgcatggtggcgtggaagtggaggtgaggacggtggtgacagtgtggtggcagcagcgacaatgatggtgatggtgatgatggtggtgatggtgatgatggtggtgatggtggtgatggtggtgatggtggtgatggtgataatggtgatggtggtgatgatggtgatggtgatgatggtggtgatggcggtggtgatggtgatggtggtgatggtgatggtggtggtggtgatgatggtggtggtggtgatggtggtggtgatgatggtgatggtgatgatggtggtggtgatggtggtgatggtgatgatggtgatggtgatggtggtggtgatagtgatgatggagatggtggtgatggtggtggtgatggtgatgatggtggtggtggtgatggtgatgatggtgatggtgatggtggtgatggtgatggtggtgatggcgatggtggtgatgatggtgatggcgatgatggtgatgatagtgatggtgatgatggtgatggtgatagtgatgataatggtgatgatggtgatggtggtggtgatggtggtggtggtgatgatagtgatggtgatgatgatggtgatgatgatggtgatgatggtgatggtgatgatgatagtgatggtggtgatggtgatggtgatgatggtgatgatagtgatggcgatgatggtgatgatagtgatggtgatgatggtgatgatgataatggtgatgatggtggtggtgatggtggtggtggtgatggtggtgatggtgatggtggtgatggcgatgatggtgatgatggtgatggcgatgatggtgatagtgatggtgatgatggtgatggtgatagtgatgataatggtgatgatgatggtgatggtgatagtgatgataatggtgatgatgatggtgatggtggtggtgatggtagtggtggtgatgatagtgatggtgatgatgatggtgatgatggtgatggtgatgatagtgatggtggtgatggtgatggtgatgatggtgatgatagtgatggcgatgatggtgatgatagtgatggtgatgatggtgatggtgatgatgatggtgatggtggtggtgatggtggtggtgatggtggtggtggtgatgatagtgatggtgatgatgataatggtgatgatggtgatggtgatgatgatgatgatagtgatggtggtgatggtgatggtggtgatgatgatgatagtgatggcgatgatggtgatgatagtgatggtgatgatgatgatagtgatggtggtgatggtgatggtgatgatagtgatggcgatgatggtgatgatagtgatggtgatgatggtgatggtgatgataatggtgatgatgatggtgatggtggtggtgatggtggtggtggtgatgatagtgatggtgatgatggtgatgataatggtgacgatggtgatgatgatgatagtgatggtggtgatggtgatggtggtgatggtgatggtggtgatgatagtgatggtgatggtgatgatggtgatggtgatgataatggtgatgatggtgatggtgatgatggtggtgatggtgatgatggaggcaatggtgatgatagtgatggtgatggcgatagtgatagtgatggtggtggtgatagtgatggtgatggtgatgatgacagtgatgatggtgatggtggtgatggaggggtgctgacagagtggtggagggatggggactgtatggaccatttttcagtctcttgatcctcaaccaccctgcatctgaccctatcatccctttgaggggagaatcccctactcaagaccagctcccatctcccactttagaagcaggaagcagcagccactcgcctccctgccttcaacagggctgagggtgaggacccaaccaccaggtgtttcaggctctggattggcggccagggctgtagggagcgggacatggcatctcagtcctggggcatggaacctcacggcttccaaggcagctgcagcgtgggtggtgccatagcatcacccctacccggcctctgtggagtggctacatggcaggcccttcatcgaggcatctccctggctgggcggcccctaaccctctcttcccccctgggaggggagtgagcacccaggcttgcatgtatccccccccatcggccagagcctgctcatttctgccaacagacagcatggcaggcagtgtctgatgctgccagtaacagaaaactggccacaggctggctcaagcagtgacactgatcatctcctgaaacgggagtccagagagccctgggcatggtgggttcccaggcagccactatcacccgctcagcagcttccccggagtcctccgttcttacctcctcaccgaaccactctcctgggtcagctctgacctcagcctgacgccctcacggtagtaatgtggctgctggtattccaggcctcacatccaggcaggacaaagtccagaggaaaaagaggcactggctctgcttgtgtcttcataggagtaagaaaacttctcccctaagtcctagcagacacttcttcacactcatttgccagaactgagtcccccaactgctcagctagcccctctggaggggggtaaaaccagtgttgcccagaccaaggcggactccactcctctcctattttgaggccatgtccccggaagcaggtggctgaatgagtagccccagacagcatcctgtctgaagggggtgtggggcaactctggggacaccaaagtgctggcctgggaggtgcagtggcggggggagccctgcgatgctgtggcttccttcagtgcccgcagggacggcgttcccacacctctcatgggcccctcctgcgggctcctgctgcccccgggtaccgtgtcagtgttgccctccactgggcccaggcagctgcttttagttcagtatttgccaggatctagagctggtggcagtggggatgctggcacgaatactcggtcacagtgcaggggacatgccgggtgctcctctgcgtctgatcagtgatgagtgtgagggagatcccagcctggggcgtgaggggcagctttggggctggcagaaggcaaaaggtcccaagctgtctggcatggtcacagcctggcatcctctcccctgggcacagcgtgggatgggatctggccccaccctcaggccctgtgggggctctgcccaccactccctcccagtccccagctggacaggccaccagagtccctgggccttgtgggaagctccgcaatctgacacaccactcccagtgtctggctgccatgcaaacagggaggtggtttgtgggaggagccagggacttagttcacagaagatcctgggtaggctctggtgcctgctgtccccatgctgggcatgggtgcccctccatcccctcgcaggaaccccagatggagcccggggcagtcttgtcctcccccaggggtcctgggagaccaagcacagatggttggggaaagctgcagaggtgacagggaccagcccctggctggagcccaggggtgccccatcaccatccgcaccatccccttcattaggtcctgcctgtgcccatccagcagcttagggtgagttataaatagaggctggggtaagccctgggtcaagagagcagggcaaggagattaccagctgattactgattagcagagagtgggggctgtgccaagcagaagggcctggctcctgggggtgtggagggaggtcagggctcccttggggacagtgtgcagggtccacagacggcacatatggccctggggcagggttcccagggtctctgagaggtgccttccaaatcttctcaagtcaagagggttctagatgagacccacctctggcttcaggggtgccccccaaaatatgccccctcccctgctccctacccaggagaggcgtgaggggcttccccatctcctccctccaggggtcaacgtctcagccaatcaggatgatgaactagaccacgagaccttcctgatgcaaattgaccaggagacaaagaagtgcaccttctattccagcactgggggctactggaccctggtcacccatgggggcattcacgccacagccacacaagtgtgagtgcacacatcccttcctcctccatcatccccatccccaccatcaccatccccatcatcaccatccccaccatccgcatccccatctccatccccaccacccccacccccaccagccccatccccatgaccaccatccccatctccaccatctccatcaccatcatcgccatccccatccccatcatcaccatccctatcaccaccatccccatcatcaccatccccaccatccgcatccccatctccatccccaccacccccaccaccaccagccccatccccatcaccaccatccccatctccaccatctccatcaccatcatcaccatccccatctccatcaccaccatccccatcaccatccccatctctatctctaccatgcccatcaccatcatcaccatccccatctccaccatccccattaccatctccaccatccccatctccatccccaccatccccatctccatccccatctctgccatccccaccatcaccatccccatctccatttacatccccatccccatccccctcaccatcctcatccccatccccctcaccatcctcatccccatctccaccatccccatctccatcaccatccccctctccatccccatccccatctccatcaccatccccctctccatccccatccccatctccatcttcaccatccccaccaccgttcccatcacctgcaccatcactcccaccaccatcactgcctcggccatgaggattgccgtagcagctcagtcagaaaggaaagcccactggggcagggtagcgcctgatggtggtgggtgtgtcagtggagggcaggcttctgtcccactccttggaacctgaggaggatggggaagtgagaccctgcacccccatctcctgctgtcctgaggagaccttttgctgctccctccagttctgccaacaccatgtttgagatggagtggcgtggccggcgggtagcactcaaagccagcaacgggcgctacgtgtgcatgaagaagaatgggcagctggcggctatcagcgattttgtcggtgagcactctgcctgccaggtactggggcaggggctgtctccacccagggaaaggacctgcccagacaccccatctccaccaagagctggaccctccccagcccacggaacgggtgctgtcatggagtcatacttgctagtcaagataactcgtcttggcaagggaaacaggtctgaatgtccttatctccgctgctgggaaccccctaggcgccttgccaaggccgcacatgaggcaatggcaggcctgggtccctaagtccaggtgtggcgtttcccagggcccccaccccgcccggcctggacagggaaggtggcgggaggggcagcgcagcagacgctctccccgccaggcaaggacgaagagttcaccctcaagctcatcaaccggcccatcctggtgctgcgcggcctggacggcttcgtctgccaccaccgcggctccaaccagctggacaccaaccgctccgtctacgacgtcttccacctgagcttcagcgacggcgcctaccggatccgaggtgcgtggcggggcgggtgggcacgcgggagcgggggtggcagcgggcaggtgggcacccccgccgacgccgtcccgtcccccaggccgcgacggagggttctggtacacgggcagccacggcagcgtgtgcagcgacggcgaacgcgccgaggacttcgtcttcgagttccgtgagcgcggccgcctggccatccgcgcccggagcggcaagtacctgcgcggcggcgcctcgggcctgctgcgggccgatgccgacgccccggccgggaccgcgctttgggagtactgaggccgcgcccagaccagcctgtcgcgcattaaaaccgtgtctctcccgca

SEQ ID NO: 2 - DNA, 8735 bp, Homo sapien
cagggggttcgtgacgccggctgggtctgggggctgtgggccagccgagccgacccgggcttctgggggaccgcgggggccgtgagcactcagagggcgcatcccaggcccctccggggacccggccagcctgaagatgccgacgaacggcctgcaccaggtgctgaagatccagtttggcctcgtcaacgacactgaccgctacctgacagctgagagcttcggcttcaaggtcaatgcctcggcacccagcctcaagaggaagcagacctgggtgctggaacccgacccaggacaaggcacggctgtgctgctccgcagcagccacctgggccgctacctgtcggcagaagaggacgggcgcgtggcctgtgaggcagagcagccgggccgtgactgccgcttcctggtcctgccgcagccagatgggcgctgggtgctgcggtccgagccgcacggccgcttcttcggaggcaccgaggaccagctgtcctgcttcgccacagccgtttccccggccgagctgtggaccgtgcacctggccatctacccgcaggcccacctgctgagcgtgagccggcggcgctacgtgcacctgtgcccgcgggaggacgagatggccgcagacggagacaagccctggggcgtggacgccctcctcaccctcatcttccggagccgacggtactgcctcaagtcctgtgacagccgctacctgcgcagcgacggccgtctggtctgggagcctgagccccgtgcctgctacacgctggagttcaaggcgggcaagctggccttcaaggactgcgacggccactacctggcacccgtggggcccgcaggcaccctcaaggccggccgaaacacgcgacctggcaaggatgagctctttgatctggaggagagtcacccacaggtggtgctggtggctgccaaccaccgctacgtctctgtgcggcaaggtagggagggcacaggtggcgacctcctgaggggtgctgggacccccctgcttcagggaggaggccgtgggggtctcacggggagtggtatcgtgtctgtgcgttcacatgtctgttctgggctgggggtccatgtgggacatgtgtggccactcagggtgtaggtgggtgggcctcgggccatgcccaggcgacccccactgaggggtggtggcttcagggtcagaggcaagggttcctggcctttctcagcatagctggagaatgtctcagccaagccctgggcagctgcggagtctgagactggagaggtgtgggccaggcgatgggcagtgcccagcaggggcaggaggcccacagcctggcctggtgccatgaggggcatgtgggcaggaggctgtggggggtccatatctccccttctttttctccaccccattttctggacttcatttatttatttattttttgagacagagtctcgctctgtcacccaggctggagcgcagtggcgtgatctcggctcactgcaagcgccgcctcacgggttcacgccattctcctgcctcagcctcccgagtagctgggactacaggcgcccgccaccacgcccggctaattttttgtattttttagaagagacggggtttcactgtgttagccaggatggtcttgatctcctgaccttgtgatctgtccacctcggcctcccaaagtgctgggattacaggcgtgagccaccgtgcccggctgcattttctggactttaaaggaaattggggaggagcccagggtagggcagggagctggggatcgggcggggatagcaccaccacgtgcctgaccagtggagcctcgtgtcctcaggagtgggggggcttaaggtcagctccagtgatggaggacacggtgggcaggcagctttacccggggcctgggctcctggtggggaggcacctccctgccccagtggggcgtggcctggctctccccagttcccaggtcaccagttgcctgtctgtgtgactccctccaccgcctatggggtgaaccccagcagttcctccttccccacaagctgagctctgagggaaaagccctggcccgggcagtcactacccacctgggctcctggctccatgcaccccagagtggctcggaggtggtctgaaaaggcgaggtggggagagccgggtgcatggagctcctcctcccaactcaggtccttccagaccagcatcagctgggcaaggagagctcccctgtctcctggcagctcccaggtgcccaccaagcccccaccctgacggatgtccaggccccctgggtacactgacactctggggccagatggcagaggccccaccctgtgcatggagaggggagcccagccatggctatggggtcctgcacctgcagttggcatcctcgggcctgtcccagcagtgacagggtcccaggagtgagaattcaactgtggatgcacggccatggcccttccttcctatcacagcccacagtccagctgtaatgcctgctggcctgggcccaggccgggcatgtggcaatccttaggtggttaaagggggtaagtgggacagtggcagtgagaatgcttcctccatggaagccaaagacactagacctttaggcatttgtatatggacagcttggaaagcagactcaaagtggcagtcatggccgtggccgtggcattgtggtgtgatgtgcatggtggcgtggaagtggaggtgaggacggtggtgacagtgtggtggcagcagcgacaatgatggtgatggtgatgatggtggtgatggtgatgatggtggtgatggtggtgatggtggtgatggtggtgatggtgataatggtgatggtggtgatgatggtgatggtgatgatggtggtgatggcggtggtgatggtgatggtggtgatggtgatggtggtggtggtgatgatggtggtggtggtgatggtggtggtgatgatggtgatggtgatgatggtggtggtgatggtggtgatggtgatgatggtgatggtgatggtggtggtgatagtgatgatggagatggtggtgatggtggtggtgatggtgatgatggtggtggtggtgatggtgatgatggtgatggtgatggtggtgatggtgatggtggtgatggcgatggtggtgatgatggtgatggcgatgatggtgatgatagtgatggtgatgatggtgatggtgatagtgatgataatggtgatgatggtgatggtggtggtgatggtggtggtggtgatgatagtgatggtgatgatgatggtgatgatgatggtgatgatggtgatggtgatgatgatagtgatggtggtgatggtgatggtgatgatggtgatgatagtgatggcgatgatggtgatgatagtgatggtgatgatggtgatgatgataatggtgatgatggtggtggtgatggtggtggtggtgatggtggtgatggtgatggtggtgatggcgatgatggtgatgatggtgatggcgatgatggtgatagtgatggtgatgatggtgatggtgatagtgatgataatggtgatgatgatggtgatggtgatagtgatgataatggtgatgatgatggtgatggtggtggtgatggtagtggtggtgatgatagtgatggtgatgatgatggtgatgatggtgatggtgatgatagtgatggtggtgatggtgatggtgatgatggtgatgatagtgatggcgatgatggtgatgatagtgatggtgatgatggtgatggtgatgatgatggtgatggtggtggtgatggtggtggtgatggtggtggtggtgatgatagtgatggtgatgatgataatggtgatgatggtgatggtgatgatgatgatgatagtgatggtggtgatggtgatggtggtgatgatgatgatagtgatggcgatgatggtgatgatagtgatggtgatgatgatgatagtgatggtggtgatggtgatggtgatgatagtgatggcgatgatggtgatgatagtgatggtgatgatggtgatggtgatgataatggtgatgatgatggtgatggtggtggtgatggtggtggtggtgatgatagtgatggtgatgatggtgatgataatggtgacgatggtgatgatgatgatagtgatggtggtgatggtgatggtggtgatggtgatggtggtgatgatagtgatggtgatggtgatgatggtgatggtgatgataatggtgatgatggtgatggtgatgatggtggtgatggtgatgatggaggcaatggtgatgatagtgatggtgatggcgatagtgatagtgatggtggtggtgatagtgatggtgatggtgatgatgacagtgatgatggtgatggtggtgatggaggggtgctgacagagtggtggagggatggggactgtatggaccatttttcagtctcttgatcctcaaccaccctgcatctgaccctatcatccctttgaggggagaatcccctactcaagaccagctcccatctcccactttagaagcaggaagcagcagccactcgcctccctgccttcaacagggctgagggtgaggacccaaccaccaggtgtttcaggctctggattggcggccagggctgtagggagcgggacatggcatctcagtcctggggcatggaacctcacggcttccaaggcagctgcagcgtgggtggtgccatagcatcacccctacccggcctctgtggagtggctacatggcaggcccttcatcgaggcatctccctggctgggcggcccctaaccctctcttcccccctgggaggggagtgagcacccaggcttgcatgtatccccccccatcggccagagcctgctcatttctgccaacagacagcatggcaggcagtgtctgatgctgccagtaacagaaaactggccacaggctggctcaagcagtgacactgatcatctcctgaaacgggagtccagagagccctgggcatggtgggttcccaggcagccactatcacccgctcagcagcttccccggagtcctccgttcttacctcctcaccgaaccactctcctgggtcagctctgacctcagcctgacgccctcacggtagtaatgtggctgctggtattccaggcctcacatccaggcaggacaaagtccagaggaaaaagaggcactggctctgcttgtgtcttcataggagtaagaaaacttctcccctaagtcctagcagacacttcttcacactcatttgccagaactgagtcccccaactgctcagctagcccctctggaggggggtaaaaccagtgttgcccagaccaaggcggactccactcctctcctattttgaggccatgtccccggaagcaggtggctgaatgagtagccccagacagcatcctgtctgaagggggtgtggggcaactctggggacaccaaagtgctggcctgggaggtgcagtggcggggggagccctgcgatgctgtggcttccttcagtgcccgcagggacggcgttcccacacctctcatgggcccctcctgcgggctcctgctgcccccgggtaccgtgtcagtgttgccctccactgggcccaggcagctgcttttagttcagtatttgccaggatctagagctggtggcagtggggatgctggcacgaatactcggtcacagtgcaggggacatgccgggtgctcctctgcgtctgatcagtgatgagtgtgagggagatcccagcctggggcgtgaggggcagctttggggctggcagaaggcaaaaggtcccaagctgtctggcatggtcacagcctggcatcctctcccctgggcacagcgtgggatgggatctggccccaccctcaggccctgtgggggctctgcccaccactccctcccagtccccagctggacaggccaccagagtccctgggccttgtgggaagctccgcaatctgacacaccactcccagtgtctggctgccatgcaaacagggaggtggtttgtgggaggagccagggacttagttcacagaagatcctgggtaggctctggtgcctgctgtccccatgctgggcatgggtgcccctccatcccctcgcaggaaccccagatggagcccggggcagtcttgtcctcccccaggggtcctgggagaccaagcacagatggttggggaaagctgcagaggtgacagggaccagcccctggctggagcccaggggtgccccatcaccatccgcaccatccccttcattaggtcctgcctgtgcccatccagcagcttagggtgagttataaatagaggctggggtaagccctgggtcaagagagcagggcaaggagattaccagctgattactgattagcagagagtgggggctgtgccaagcagaagggcctggctcctgggggtgtggagggaggtcagggctcccttggggacagtgtgcagggtccacagacggcacatatggccctggggcagggttcccagggtctctgagaggtgccttccaaatcttctcaagtcaagagggttctagatgagacccacctctggcttcaggggtgccccccaaaatatgccccctcccctgctccctacccaggagaggcgtgaggggcttccccatctcctccctccaggggtcaacgtctcagccaatcaggatgatgaactagaccacgagaccttcctgatgcaaattgaccaggagacaaagaagtgcaccttctattccagcactgggggctactggaccctggtcacccatgggggcattcacgccacagccacacaagtgtgagtgcacacatcccttcctcctccatcatccccatccccaccatcaccatccccatcatcaccatccccaccatccgcatccccatctccatccccaccacccccacccccaccagccccatccccatgaccaccatccccatctccaccatctccatcaccatcatcgccatccccatccccatcatcaccatccctatcaccaccatccccatcatcaccatccccaccatccgcatccccatctccatccccaccacccccaccaccaccagccccatccccatcaccaccatccccatctccaccatctccatcaccatcatcaccatccccatctccatcaccaccatccccatcaccatccccatctctatctctaccatgcccatcaccatcatcaccatccccatctccaccatccccattaccatctccaccatccccatctccatccccaccatccccatctccatccccatctctgccatccccaccatcaccatccccatctccatttacatccccatccccatccccctcaccatcctcatccccatccccctcaccatcctcatccccatctccaccatccccatctccatcaccatccccctctccatccccatccccatctccatcaccatccccctctccatccccatccccatctccatcttcaccatccccaccaccgttcccatcacctgcaccatcactcccaccaccatcactgcctcggccatgaggattgccgtagcagctcagtcagaaaggaaagcccactggggcagggtagcgcctgatggtggtgggtgtgtcagtggagggcaggcttctgtcccactccttggaacctgaggaggatggggaagtgagaccctgcacccccatctcctgctgtcctgaggagaccttttgctgctccctccagttctgccaacaccatgtttgagatggagtggcgtggccggcgggtagcactcaaagccagcaacgggcgctacgtgtgcatgaagaagaatgggcagctggcggctatcagcgattttgtcggtgagcactctgcctgccaggtactggggcaggggctgtctccacccagggaaaggacctgcccagacaccccatctccaccaagagctggaccctccccagcccacggaacgggtgctgtcatggagtcatacttgctagtcaagataactcgtcttggcaagggaaacaggtctgaatgtccttatctccgctgctgggaaccccctaggcgccttgccaaggccgcacatgaggcaatggcaggcctgggtccctaagtccaggtgtggcgtttcccagggcccccaccccgcccggcctggacagggaaggtggcgggaggggcagcgcagcagacgctctccccgccaggcaaggacgaagagttcaccctcaagctcatcaaccggcccatcctggtgctgcgcggcctggacggcttcgtctgccaccaccgcggctccaaccagctggacaccaaccgctccgtctacgacgtcttccacctgagcttcagcgacggcgcctaccggatccgaggtgcgtggcggggcgggtgggcacgcgggagcgggggtggcagcgggcaggtgggcacccccgccgacgccgtcccgtcccccaggccgcgacggagggttctggtacacgggcagccacggcagcgtgtgcagcgacggcgaacgcgccgaggacttcgtcttcgagttccgtgagcgcggccgcctggccatccgcgcccggagcggcaagtacctgcgcggcggcgcctcgggcctgctgcgggccgatgccgacgccccggccgggaccgcgctttgggagtactgaggccgcgcccagaccagcctgtcgcgcattaaaaccgtgtctctcccgca

SEQ ID NO: 3 - DNA, 1720 bp, Homo sapien
caggggguucgugacgccggcugggucugggggcugugggccagccgagccgacccgggcuucugggggaccgcgggggccgugagcacucagagggugcaucccaggccccuccggggacccggccagccugaagaugccgacgaacggccugcaccaggugcugaagauccaguuuggccucgucaacgacacugaccgcuaccugacagcugagagcuucggcuucaaggucaaugccucggcacccagccucaagaggaagcagaccugggugcuggaacccgacccaggacaaggcacggcugugcugcuccgcagcagccaccugggccgcuaccugucggcagaagaggacgggcgcguggccugugaggcagagcagccgggccgugacugccgcuuccugguccugccgcagccagaugggcgcugggugcugcgguccgagccgcacggccgcuucuucggaggcaccgaggaccagcuguccugcuucgccacagccguuuccccggccgagcuguggaccgugcaccuggccauccacccgcaggcccaccugcugagcgugagccggcggcgcuacgugcaccugugcccgcgggaggacgagauggccgcagacggagacaagcccuggggcguggacgcccuccucacccucaucuuccggagccgacgguacugccucaaguccugugacagccgcuaccugcgcagcgacggccgucuggucugggagccugagccccgugccugcuacacgcuggaguucaaggcgggcaagcuggccuucaaggacugcgacggccacuaccuggcacccguggggcccgcaggcacccucaaggccggccgaaacacgcgaccuggcaaggaugagcucuuugaucuggaggagagucacccacagguggugcugguggcugccaaccaccgcuacgucucugugcggcaaggggucaacgucucagccaaucaggaugaugaacuagaccacgagaccuuccugaugcaaauugaccaggagacaaagaagugcaccuucuauuccagcacugggggcuacuggacccuggucacccaugggggcauucacgccacagccacacaaguuucugccaacaccauguuugagauggaguggcguggccggcggguagcacucaaagccagcaacgggcgcuacgugugcaugaagaagaaugggcagcuggcggcuaucagcgauuuugucggcaaggacgaagaguucacccucaagcucaucaaccggcccauccuggugcugcgcggccuggacggcuucgucugccaccaccgcggcuccaaccagcuggacaccaaccgcuccgucuacgacgucuuccaccugagcuucagcgacggcgccuaccggauccgaggccgcgacggaggguucugguacacgggcagccacggcagcgugugcagcgacggcgaacgcgccgaggacuucgucuucgaguuccgugagcgcggccgccuggccauccgcgcccggagcggcaaguaccugcgcggcggcgccucgggccugcugcgggccgaugccgacgccccggccgggaccgcgcuuugggaguacugaggccgcgcccagaccagccugucgcgcauuaaaaccgugucucucccgcaaaaaaaaaaaaaaaaaaaaaaaaaaaaaaaaaaaaaaaaaaaaaaaaaaaaaaaa

SEQ ID NO: 4 - DNA, 1577 bp, Homo sapien
ccgugagcacucagagggugcaucccaggccccuccggggacccggccagccugaagaugccgacgaacggccugcaccaggugcugaagauccaguuuggccucgucaacgacacugaccgcuaccugacagcugagagcuucggcuucaaggucaaugccucggcacccagccucaagaggaagcagaccugggugcuggaacccgacccaggacaaggcacggcugugcugcuccgcagcagccaccugggccgcuaccugucggcagaagaggacgggcgcguggccugugaggcagagcagccgggccgugacugccgcuuccugguccugccgcagccagaugggcgcugggugcugcgguccgagccgcacggccgcuucuucggaggcaccgaggaccagcuguccugcuucgccacagccguuuccccggccgagcuguggaccgugcaccuggccauccacccgcaggcccaccugcugagcgugagccggcggcgcuacgugcaccugugcccgcgggaggacgagauggccgcagacggagacaagcccuggggcguggacgcccuccucacccucaucuuccggagccgacgguacugccucaaguccugugacagccgcuaccugcgcagcgacggccgucuggucugggagccugagccccgugccugcuacacgcuggaguucaaggcgggcaagcuggccuucaaggacugcgacggccacuaccuggcacccguggggcccgcaggcacccucaaggccggccgaaacacgcgaccuggcaaggaugagcucuuugaucuggaggagagucacccacagguggugcugguggcugccaaccaccgcuacgucucugugcggcaaggggucaacgucucagccaaucaggaugaugaacuagaccacgagaccuuccugaugcaaauugaccaggagacaaagaagugcaccuucuauuccagcacugggggcuacuggacccuggucacccaugggggcauucacgccacagccacacaaguuucugccaacaccauguuugagauggaguggcguggccggcggguagcacucaaagccagcaacgggcgcuacgugugcaugaagaagaaugggcagcuggcggcuaucagcgauuuugucggcaaggacgaagaguucacccucaagcucaucaaccggcccauccuggugcugcgcggccuggacggcuucgucugccaccaccgcggcuccaaccagcuggacaccaaccgcuccgucuacgacgucuuccaccugagcuucagcgacggcgccuaccggauccgaggccgcgacggaggguucugguacacgggcagccacggcagcgugugcagcgacggcgaacgcgccgaggacuucgucuucgaguuccgugagcgcggccgccuggccauccgcgcccggagcggcaaguaccugcgcggcggcgccucgggccugcugcgggccgaugccgacgccccggccgggaccgcgcuuugggaguacugaggccgcgcccagaccagccugucgcgcauuaaaaccguguc

SEQ ID NO: 5 - DNA, 1762 bp, Homo sapien
gcaggcaggggguucgugacgccggcugggucugggggcugugggccagccgagccgacccgggcuucugggggaccgcgggggccgugagcacucagagggcgcaucccaggccccuccggggacccggccagccugaagaugccgacgaacggccugcaccaggugcugaagauccaguuuggccucgucaacgacacugaccgcuaccugacagcugagagcuucggcuucaaggucaaugccucggcacccagccucaagaggaagcagaccugggugcuggaacccgacccaggacaaggcacggcugugcugcuccgcagcagccaccugggccgcuaccugucggcagaagaggacgggcgcguggccugugaggcagagcagccgggccgugacugccgcuuccugguccugccgcagccagaugggcgcugggugcugcgguccgagccgcacggccgcuucuucggaggcaccgaggaccagcuguccugcuucgccacagccguuuccccggccgagcuguggaccgugcaccuggccauccacccgcaggcccaccugcugagcgugagccggcggcgcuacgugcaccugugcccgcgggaggacgagauggccgcagacggagacaagcccuggggcguggacgcccuccucacccucaucuuccggagccgacgguacugccucaaguccugugacagccgcuaccugcgcagcgacggccgucuggucugggagccugagccccgugccugcuacacgcuggaguucaaggcgggcaagcuggccuucaaggacugcgacggccacuaccuggcacccguggggcccgcaggcacccucaaggccggccgaaacacgcgaccuggcaaggaugagcucuuugaucuggaggagagucacccacagguggugcugguggcugccaaccaccgcuacgucucugugcggcaaggggucaacgucucagccaaucaggaugaugaacuagaccacgagaccuuccugaugcaaauugaccaggagacaaagaagugcaccuucuauuccagcacugggggcuacuggacccuggucacccaugggggcauucacgccacagccacacaaguuucugccaacaccauguuugagauggaguggcguggccggcggguagcacucaaagccagcaacgggcgcuacgugugcaugaagaagaaugggcagcuggcggcuaucagcgauuuugucgggcccccaccccgcccggccuggacagggaagguggcgggaggggcagcgcagcagacgcucuccccgccaggcaaggacgaagaguucacccucaagcucaucaaccggcccauccuggugcugcgcggccuggacggcuucgucugccaccaccgcggcuccaaccagcuggacaccaaccgcuccgucuacgacgucuuccaccugagcuucagcgacggcgccuaccggauccgaggccgcgacggaggguucugguacacgggcagccacggcagcgugugcagcgacggcgaacgcgccgaggacuucgucuucgaguuccgugagcgcggccgccuggccauccgcgcccggagcggcaaguaccugcgcggcggcgccucgggccugcugcgggccgaugccgacgccccggccgggaccgcgcuuugggaguacugaggccgcgcccagaccagccugucgcgcauuaaaaccgugucucucccgcaaaaaaaaaaaaaaaaaaaaa

SEQ ID NO: 6 - DNA, 1720 bp, Homo sapien
caggggguucgugacgccggcugggucugggggcugugggccagccgagccgacccgggcuucugggggaccgcgggggccgugagcacucagagggugcaucccaggccccuccggggacccggccagccugaagaugccgacgaacggccugcaccaggugcugaagauccaguuuggccucgucaacgacacugaccgcuaccugacagcugagagcuucggcuucaaggucaaugccucggcacccagccucaagaggaagcagaccugggugcuggaacccgacccaggacaaggcacggcugugcugcuccgcagcagccaccugggccgcuaccugucggcagaagaggacgggcgcguggccugugaggcagagcagccgggccgugacugccgcuuccugguccugccgcagccagaugggcgcugggugcugcgguccgagccgcacggccgcuucuucggaggcaccgaggaccagcuguccugcuucgccacagccguuuccccggccgagcuguggaccgugcaccuggccaucuacccgcaggcccaccugcugagcgugagccggcggcgcuacgugcaccugugcccgcgggaggacgagauggccgcagacggagacaagcccuggggcguggacgcccuccucacccucaucuuccggagccgacgguacugccucaaguccugugacagccgcuaccugcgcagcgacggccgucuggucugggagccugagccccgugccugcuacacgcuggaguucaaggcgggcaagcuggccuucaaggacugcgacggccacuaccuggcacccguggggcccgcaggcacccucaaggccggccgaaacacgcgaccuggcaaggaugagcucuuugaucuggaggagagucacccacagguggugcugguggcugccaaccaccgcuacgucucugugcggcaaggggucaacgucucagccaaucaggaugaugaacuagaccacgagaccuuccugaugcaaauugaccaggagacaaagaagugcaccuucuauuccagcacugggggcuacuggacccuggucacccaugggggcauucacgccacagccacacaaguuucugccaacaccauguuugagauggaguggcguggccggcggguagcacucaaagccagcaacgggcgcuacgugugcaugaagaagaaugggcagcuggcggcuaucagcgauuuugucggcaaggacgaagaguucacccucaagcucaucaaccggcccauccuggugcugcgcggccuggacggcuucgucugccaccaccgcggcuccaaccagcuggacaccaaccgcuccgucuacgacgucuuccaccugagcuucagcgacggcgccuaccggauccgaggccgcgacggaggguucugguacacgggcagccacggcagcgugugcagcgacggcgaacgcgccgaggacuucgucuucgaguuccgugagcgcggccgccuggccauccgcgcccggagcggcaaguaccugcgcggcggcgccucgggccugcugcgggccgaugccgacgccccggccgggaccgcgcuuugggaguacugaggccgcgcccagaccagccugucgcgcauuaaaaccgugucucucccgcaaaaaaaaaaaaaaaaaaaaaaaaaaaaaaaaaaaaaaaaaaaaaaaaaaaaaaaa

SEQ ID NO: 7 - DNA, 1577 bp, Homo sapien
ccgugagcacucagagggugcaucccaggccccuccggggacccggccagccugaagaugccgacgaacggccugcaccaggugcugaagauccaguuuggccucgucaacgacacugaccgcuaccugacagcugagagcuucggcuucaaggucaaugccucggcacccagccucaagaggaagcagaccugggugcuggaacccgacccaggacaaggcacggcugugcugcuccgcagcagccaccugggccgcuaccugucggcagaagaggacgggcgcguggccugugaggcagagcagccgggccgugacugccgcuuccugguccugccgcagccagaugggcgcugggugcugcgguccgagccgcacggccgcuucuucggaggcaccgaggaccagcuguccugcuucgccacagccguuuccccggccgagcuguggaccgugcaccuggccaucuacccgcaggcccaccugcugagcgugagccggcggcgcuacgugcaccugugcccgcgggaggacgagauggccgcagacggagacaagcccuggggcguggacgcccuccucacccucaucuuccggagccgacgguacugccucaaguccugugacagccgcuaccugcgcagcgacggccgucuggucugggagccugagccccgugccugcuacacgcuggaguucaaggcgggcaagcuggccuucaaggacugcgacggccacuaccuggcacccguggggcccgcaggcacccucaaggccggccgaaacacgcgaccuggcaaggaugagcucuuugaucuggaggagagucacccacagguggugcugguggcugccaaccaccgcuacgucucugugcggcaaggggucaacgucucagccaaucaggaugaugaacuagaccacgagaccuuccugaugcaaauugaccaggagacaaagaagugcaccuucuauuccagcacugggggcuacuggacccuggucacccaugggggcauucacgccacagccacacaaguuucugccaacaccauguuugagauggaguggcguggccggcggguagcacucaaagccagcaacgggcgcuacgugugcaugaagaagaaugggcagcuggcggcuaucagcgauuuugucggcaaggacgaagaguucacccucaagcucaucaaccggcccauccuggugcugcgcggccuggacggcuucgucugccaccaccgcggcuccaaccagcuggacaccaaccgcuccgucuacgacgucuuccaccugagcuucagcgacggcgccuaccggauccgaggccgcgacggaggguucugguacacgggcagccacggcagcgugugcagcgacggcgaacgcgccgaggacuucgucuucgaguuccgugagcgcggccgccuggccauccgcgcccggagcggcaaguaccugcgcggcggcgccucgggccugcugcgggccgaugccgacgccccggccgggaccgcgcuuugggaguacugaggccgcgcccagaccagccugucgcgcauuaaaaccguguc

SEQ ID NO: 8 - DNA, 1762 bp, Homo sapien
gcaggcaggggguucgugacgccggcugggucugggggcugugggccagccgagccgacccgggcuucugggggaccgcgggggccgugagcacucagagggcgcaucccaggccccuccggggacccggccagccugaagaugccgacgaacggccugcaccaggugcugaagauccaguuuggccucgucaacgacacugaccgcuaccugacagcugagagcuucggcuucaaggucaaugccucggcacccagccucaagaggaagcagaccugggugcuggaacccgacccaggacaaggcacggcugugcugcuccgcagcagccaccugggccgcuaccugucggcagaagaggacgggcgcguggccugugaggcagagcagccgggccgugacugccgcuuccugguccugccgcagccagaugggcgcugggugcugcgguccgagccgcacggccgcuucuucggaggcaccgaggaccagcuguccugcuucgccacagccguuuccccggccgagcuguggaccgugcaccuggccaucuacccgcaggcccaccugcugagcgugagccggcggcgcuacgugcaccugugcccgcgggaggacgagauggccgcagacggagacaagcccuggggcguggacgcccuccucacccucaucuuccggagccgacgguacugccucaaguccugugacagccgcuaccugcgcagcgacggccgucuggucugggagccugagccccgugccugcuacacgcuggaguucaaggcgggcaagcuggccuucaaggacugcgacggccacuaccuggcacccguggggcccgcaggcacccucaaggccggccgaaacacgcgaccuggcaaggaugagcucuuugaucuggaggagagucacccacagguggugcugguggcugccaaccaccgcuacgucucugugcggcaaggggucaacgucucagccaaucaggaugaugaacuagaccacgagaccuuccugaugcaaauugaccaggagacaaagaagugcaccuucuauuccagcacugggggcuacuggacccuggucacccaugggggcauucacgccacagccacacaaguuucugccaacaccauguuugagauggaguggcguggccggcggguagcacucaaagccagcaacgggcgcuacgugugcaugaagaagaaugggcagcuggcggcuaucagcgauuuugucgggcccccaccccgcccggccuggacagggaagguggcgggaggggcagcgcagcagacgcucuccccgccaggcaaggacgaagaguucacccucaagcucaucaaccggcccauccuggugcugcgcggccuggacggcuucgucugccaccaccgcggcuccaaccagcuggacaccaaccgcuccgucuacgacgucuuccaccugagcuucagcgacggcgccuaccggauccgaggccgcgacggaggguucugguacacgggcagccacggcagcgugugcagcgacggcgaacgcgccgaggacuucgucuucgaguuccgugagcgcggccgccuggccauccgcgcccggagcggcaaguaccugcgcggcggcgccucgggccugcugcgggccgaugccgacgccccggccgggaccgcgcuuugggaguacugaggccgcgcccagaccagccugucgcgcauuaaaaccgugucucucccgcaaaaaaaaaaaaaaaaaaaaa

SEQ ID NO: 9 - DNA, 1720 bp, Homo sapien
cagggggttcgtgacgccggctgggtctgggggctgtgggccagccgagccgacccgggcttctgggggaccgcgggggccgtgagcactcagagggtgcatcccaggcccctccggggacccggccagcctgaagatgccgacgaacggcctgcaccaggtgctgaagatccagtttggcctcgtcaacgacactgaccgctacctgacagctgagagcttcggcttcaaggtcaatgcctcggcacccagcctcaagaggaagcagacctgggtgctggaacccgacccaggacaaggcacggctgtgctgctccgcagcagccacctgggccgctacctgtcggcagaagaggacgggcgcgtggcctgtgaggcagagcagccgggccgtgactgccgcttcctggtcctgccgcagccagatgggcgctgggtgctgcggtccgagccgcacggccgcttcttcggaggcaccgaggaccagctgtcctgcttcgccacagccgtttccccggccgagctgtggaccgtgcacctggccatccacccgcaggcccacctgctgagcgtgagccggcggcgctacgtgcacctgtgcccgcgggaggacgagatggccgcagacggagacaagccctggggcgtggacgccctcctcaccctcatcttccggagccgacggtactgcctcaagtcctgtgacagccgctacctgcgcagcgacggccgtctggtctgggagcctgagccccgtgcctgctacacgctggagttcaaggcgggcaagctggccttcaaggactgcgacggccactacctggcacccgtggggcccgcaggcaccctcaaggccggccgaaacacgcgacctggcaaggatgagctctttgatctggaggagagtcacccacaggtggtgctggtggctgccaaccaccgctacgtctctgtgcggcaaggggtcaacgtctcagccaatcaggatgatgaactagaccacgagaccttcctgatgcaaattgaccaggagacaaagaagtgcaccttctattccagcactgggggctactggaccctggtcacccatgggggcattcacgccacagccacacaagtttctgccaacaccatgtttgagatggagtggcgtggccggcgggtagcactcaaagccagcaacgggcgctacgtgtgcatgaagaagaatgggcagctggcggctatcagcgattttgtcggcaaggacgaagagttcaccctcaagctcatcaaccggcccatcctggtgctgcgcggcctggacggcttcgtctgccaccaccgcggctccaaccagctggacaccaaccgctccgtctacgacgtcttccacctgagcttcagcgacggcgcctaccggatccgaggccgcgacggagggttctggtacacgggcagccacggcagcgtgtgcagcgacggcgaacgcgccgaggacttcgtcttcgagttccgtgagcgcggccgcctggccatccgcgcccggagcggcaagtacctgcgcggcggcgcctcgggcctgctgcgggccgatgccgacgccccggccgggaccgcgctttgggagtactgaggccgcgcccagaccagcctgtcgcgcattaaaaccgtgtctctcccgcaaaaaaaaaaaaaaaaaaaaaaaaaaaaaaaaaaaaaaaaaaaaaaaaaaaaaaaa

SEQ ID NO: 10 - DNA, 1577 bp, Homo sapien
ccgtgagcactcagagggtgcatcccaggcccctccggggacccggccagcctgaagatgccgacgaacggcctgcaccaggtgctgaagatccagtttggcctcgtcaacgacactgaccgctacctgacagctgagagcttcggcttcaaggtcaatgcctcggcacccagcctcaagaggaagcagacctgggtgctggaacccgacccaggacaaggcacggctgtgctgctccgcagcagccacctgggccgctacctgtcggcagaagaggacgggcgcgtggcctgtgaggcagagcagccgggccgtgactgccgcttcctggtcctgccgcagccagatgggcgctgggtgctgcggtccgagccgcacggccgcttcttcggaggcaccgaggaccagctgtcctgcttcgccacagccgtttccccggccgagctgtggaccgtgcacctggccatccacccgcaggcccacctgctgagcgtgagccggcggcgctacgtgcacctgtgcccgcgggaggacgagatggccgcagacggagacaagccctggggcgtggacgccctcctcaccctcatcttccggagccgacggtactgcctcaagtcctgtgacagccgctacctgcgcagcgacggccgtctggtctgggagcctgagccccgtgcctgctacacgctggagttcaaggcgggcaagctggccttcaaggactgcgacggccactacctggcacccgtggggcccgcaggcaccctcaaggccggccgaaacacgcgacctggcaaggatgagctctttgatctggaggagagtcacccacaggtggtgctggtggctgccaaccaccgctacgtctctgtgcggcaaggggtcaacgtctcagccaatcaggatgatgaactagaccacgagaccttcctgatgcaaattgaccaggagacaaagaagtgcaccttctattccagcactgggggctactggaccctggtcacccatgggggcattcacgccacagccacacaagtttctgccaacaccatgtttgagatggagtggcgtggccggcgggtagcactcaaagccagcaacgggcgctacgtgtgcatgaagaagaatgggcagctggcggctatcagcgattttgtcggcaaggacgaagagttcaccctcaagctcatcaaccggcccatcctggtgctgcgcggcctggacggcttcgtctgccaccaccgcggctccaaccagctggacaccaaccgctccgtctacgacgtcttccacctgagcttcagcgacggcgcctaccggatccgaggccgcgacggagggttctggtacacgggcagccacggcagcgtgtgcagcgacggcgaacgcgccgaggacttcgtcttcgagttccgtgagcgcggccgcctggccatccgcgcccggagcggcaagtacctgcgcggcggcgcctcgggcctgctgcgggccgatgccgacgccccggccgggaccgcgctttgggagtactgaggccgcgcccagaccagcctgtcgcgcattaaaaccgtgtc

SEQ ID NO: 11 - DNA, 1762 bp, Homo sapien
gcaggcagggggttcgtgacgccggctgggtctgggggctgtgggccagccgagccgacccgggcttctgggggaccgcgggggccgtgagcactcagagggcgcatcccaggcccctccggggacccggccagcctgaagatgccgacgaacggcctgcaccaggtgctgaagatccagtttggcctcgtcaacgacactgaccgctacctgacagctgagagcttcggcttcaaggtcaatgcctcggcacccagcctcaagaggaagcagacctgggtgctggaacccgacccaggacaaggcacggctgtgctgctccgcagcagccacctgggccgctacctgtcggcagaagaggacgggcgcgtggcctgtgaggcagagcagccgggccgtgactgccgcttcctggtcctgccgcagccagatgggcgctgggtgctgcggtccgagccgcacggccgcttcttcggaggcaccgaggaccagctgtcctgcttcgccacagccgtttccccggccgagctgtggaccgtgcacctggccatccacccgcaggcccacctgctgagcgtgagccggcggcgctacgtgcacctgtgcccgcgggaggacgagatggccgcagacggagacaagccctggggcgtggacgccctcctcaccctcatcttccggagccgacggtactgcctcaagtcctgtgacagccgctacctgcgcagcgacggccgtctggtctgggagcctgagccccgtgcctgctacacgctggagttcaaggcgggcaagctggccttcaaggactgcgacggccactacctggcacccgtggggcccgcaggcaccctcaaggccggccgaaacacgcgacctggcaaggatgagctctttgatctggaggagagtcacccacaggtggtgctggtggctgccaaccaccgctacgtctctgtgcggcaaggggtcaacgtctcagccaatcaggatgatgaactagaccacgagaccttcctgatgcaaattgaccaggagacaaagaagtgcaccttctattccagcactgggggctactggaccctggtcacccatgggggcattcacgccacagccacacaagtttctgccaacaccatgtttgagatggagtggcgtggccggcgggtagcactcaaagccagcaacgggcgctacgtgtgcatgaagaagaatgggcagctggcggctatcagcgattttgtcgggcccccaccccgcccggcctggacagggaaggtggcgggaggggcagcgcagcagacgctctccccgccaggcaaggacgaagagttcaccctcaagctcatcaaccggcccatcctggtgctgcgcggcctggacggcttcgtctgccaccaccgcggctccaaccagctggacaccaaccgctccgtctacgacgtcttccacctgagcttcagcgacggcgcctaccggatccgaggccgcgacggagggttctggtacacgggcagccacggcagcgtgtgcagcgacggcgaacgcgccgaggacttcgtcttcgagttccgtgagcgcggccgcctggccatccgcgcccggagcggcaagtacctgcgcggcggcgcctcgggcctgctgcgggccgatgccgacgccccggccgggaccgcgctttgggagtactgaggccgcgcccagaccagcctgtcgcgcattaaaaccgtgtctctcccgcaaaaaaaaaaaaaaaaaaaaa

SEQ ID NO: 12 - DNA, 1720 bp, Homo sapien
cagggggttcgtgacgccggctgggtctgggggctgtgggccagccgagccgacccgggcttctgggggaccgcgggggccgtgagcactcagagggtgcatcccaggcccctccggggacccggccagcctgaagatgccgacgaacggcctgcaccaggtgctgaagatccagtttggcctcgtcaacgacactgaccgctacctgacagctgagagcttcggcttcaaggtcaatgcctcggcacccagcctcaagaggaagcagacctgggtgctggaacccgacccaggacaaggcacggctgtgctgctccgcagcagccacctgggccgctacctgtcggcagaagaggacgggcgcgtggcctgtgaggcagagcagccgggccgtgactgccgcttcctggtcctgccgcagccagatgggcgctgggtgctgcggtccgagccgcacggccgcttcttcggaggcaccgaggaccagctgtcctgcttcgccacagccgtttccccggccgagctgtggaccgtgcacctggccatctacccgcaggcccacctgctgagcgtgagccggcggcgctacgtgcacctgtgcccgcgggaggacgagatggccgcagacggagacaagccctggggcgtggacgccctcctcaccctcatcttccggagccgacggtactgcctcaagtcctgtgacagccgctacctgcgcagcgacggccgtctggtctgggagcctgagccccgtgcctgctacacgctggagttcaaggcgggcaagctggccttcaaggactgcgacggccactacctggcacccgtggggcccgcaggcaccctcaaggccggccgaaacacgcgacctggcaaggatgagctctttgatctggaggagagtcacccacaggtggtgctggtggctgccaaccaccgctacgtctctgtgcggcaaggggtcaacgtctcagccaatcaggatgatgaactagaccacgagaccttcctgatgcaaattgaccaggagacaaagaagtgcaccttctattccagcactgggggctactggaccctggtcacccatgggggcattcacgccacagccacacaagtttctgccaacaccatgtttgagatggagtggcgtggccggcgggtagcactcaaagccagcaacgggcgctacgtgtgcatgaagaagaatgggcagctggcggctatcagcgattttgtcggcaaggacgaagagttcaccctcaagctcatcaaccggcccatcctggtgctgcgcggcctggacggcttcgtctgccaccaccgcggctccaaccagctggacaccaaccgctccgtctacgacgtcttccacctgagcttcagcgacggcgcctaccggatccgaggccgcgacggagggttctggtacacgggcagccacggcagcgtgtgcagcgacggcgaacgcgccgaggacttcgtcttcgagttccgtgagcgcggccgcctggccatccgcgcccggagcggcaagtacctgcgcggcggcgcctcgggcctgctgcgggccgatgccgacgccccggccgggaccgcgctttgggagtactgaggccgcgcccagaccagcctgtcgcgcattaaaaccgtgtctctcccgcaaaaaaaaaaaaaaaaaaaaaaaaaaaaaaaaaaaaaaaaaaaaaaaaaaaaaaaa

SEQ ID NO: 13 - DNA, 1577 bp, Homo sapien
ccgtgagcactcagagggtgcatcccaggcccctccggggacccggccagcctgaagatgccgacgaacggcctgcaccaggtgctgaagatccagtttggcctcgtcaacgacactgaccgctacctgacagctgagagcttcggcttcaaggtcaatgcctcggcacccagcctcaagaggaagcagacctgggtgctggaacccgacccaggacaaggcacggctgtgctgctccgcagcagccacctgggccgctacctgtcggcagaagaggacgggcgcgtggcctgtgaggcagagcagccgggccgtgactgccgcttcctggtcctgccgcagccagatgggcgctgggtgctgcggtccgagccgcacggccgcttcttcggaggcaccgaggaccagctgtcctgcttcgccacagccgtttccccggccgagctgtggaccgtgcacctggccatctacccgcaggcccacctgctgagcgtgagccggcggcgctacgtgcacctgtgcccgcgggaggacgagatggccgcagacggagacaagccctggggcgtggacgccctcctcaccctcatcttccggagccgacggtactgcctcaagtcctgtgacagccgctacctgcgcagcgacggccgtctggtctgggagcctgagccccgtgcctgctacacgctggagttcaaggcgggcaagctggccttcaaggactgcgacggccactacctggcacccgtggggcccgcaggcaccctcaaggccggccgaaacacgcgacctggcaaggatgagctctttgatctggaggagagtcacccacaggtggtgctggtggctgccaaccaccgctacgtctctgtgcggcaaggggtcaacgtctcagccaatcaggatgatgaactagaccacgagaccttcctgatgcaaattgaccaggagacaaagaagtgcaccttctattccagcactgggggctactggaccctggtcacccatgggggcattcacgccacagccacacaagtttctgccaacaccatgtttgagatggagtggcgtggccggcgggtagcactcaaagccagcaacgggcgctacgtgtgcatgaagaagaatgggcagctggcggctatcagcgattttgtcggcaaggacgaagagttcaccctcaagctcatcaaccggcccatcctggtgctgcgcggcctggacggcttcgtctgccaccaccgcggctccaaccagctggacaccaaccgctccgtctacgacgtcttccacctgagcttcagcgacggcgcctaccggatccgaggccgcgacggagggttctggtacacgggcagccacggcagcgtgtgcagcgacggcgaacgcgccgaggacttcgtcttcgagttccgtgagcgcggccgcctggccatccgcgcccggagcggcaagtacctgcgcggcggcgcctcgggcctgctgcgggccgatgccgacgccccggccgggaccgcgctttgggagtactgaggccgcgcccagaccagcctgtcgcgcattaaaaccgtgtc

SEQ ID NO: 14 - DNA, 1762 bp, Homo sapien
gcaggcagggggttcgtgacgccggctgggtctgggggctgtgggccagccgagccgacccgggcttctgggggaccgcgggggccgtgagcactcagagggcgcatcccaggcccctccggggacccggccagcctgaagatgccgacgaacggcctgcaccaggtgctgaagatccagtttggcctcgtcaacgacactgaccgctacctgacagctgagagcttcggcttcaaggtcaatgcctcggcacccagcctcaagaggaagcagacctgggtgctggaacccgacccaggacaaggcacggctgtgctgctccgcagcagccacctgggccgctacctgtcggcagaagaggacgggcgcgtggcctgtgaggcagagcagccgggccgtgactgccgcttcctggtcctgccgcagccagatgggcgctgggtgctgcggtccgagccgcacggccgcttcttcggaggcaccgaggaccagctgtcctgcttcgccacagccgtttccccggccgagctgtggaccgtgcacctggccatctacccgcaggcccacctgctgagcgtgagccggcggcgctacgtgcacctgtgcccgcgggaggacgagatggccgcagacggagacaagccctggggcgtggacgccctcctcaccctcatcttccggagccgacggtactgcctcaagtcctgtgacagccgctacctgcgcagcgacggccgtctggtctgggagcctgagccccgtgcctgctacacgctggagttcaaggcgggcaagctggccttcaaggactgcgacggccactacctggcacccgtggggcccgcaggcaccctcaaggccggccgaaacacgcgacctggcaaggatgagctctttgatctggaggagagtcacccacaggtggtgctggtggctgccaaccaccgctacgtctctgtgcggcaaggggtcaacgtctcagccaatcaggatgatgaactagaccacgagaccttcctgatgcaaattgaccaggagacaaagaagtgcaccttctattccagcactgggggctactggaccctggtcacccatgggggcattcacgccacagccacacaagtttctgccaacaccatgtttgagatggagtggcgtggccggcgggtagcactcaaagccagcaacgggcgctacgtgtgcatgaagaagaatgggcagctggcggctatcagcgattttgtcgggcccccaccccgcccggcctggacagggaaggtggcgggaggggcagcgcagcagacgctctccccgccaggcaaggacgaagagttcaccctcaagctcatcaaccggcccatcctggtgctgcgcggcctggacggcttcgtctgccaccaccgcggctccaaccagctggacaccaaccgctccgtctacgacgtcttccacctgagcttcagcgacggcgcctaccggatccgaggccgcgacggagggttctggtacacgggcagccacggcagcgtgtgcagcgacggcgaacgcgccgaggacttcgtcttcgagttccgtgagcgcggccgcctggccatccgcgcccggagcggcaagtacctgcgcggcggcgcctcgggcctgctgcgggccgatgccgacgccccggccgggaccgcgctttgggagtactgaggccgcgcccagaccagcctgtcgcgcattaaaaccgtgtctctcccgcaaaaaaaaaaaaaaaaaaaaa

SEQ ID NO: 15 - protein, 492 aa, Homo sapien
MPTNGLHQVLKIQFGLVNDTDRYLTAESFGFKVNASAPSLKRKQTWVLEPDPGQGTAVLLRSSHLGRYLSAEEDGRVACEAEQPGRDCRFLVLPQPDGRWVLRSEPHGRFFGGTEDQLSCFATAVSPAELWTVHLAIHPQAHLLSVSRRRYVHLCPREDEMAADGDKPWGVDALLTLIFRSRRYCLKSCDSRYLRSDGRLVWEPEPRACYTLEFKAGKLAFKDCDGHYLAPVGPAGTLKAGRNTRPGKDELFDLEESHPQVVLVAANHRYVSVRQGVNVSANQDDELDHETFLMQIDQETKKCTFYSSTGGYWTLVTHGGIHATATQVSANTMFEMEWRGRRVALKASNGRYVCMKKNGQLAAISDFVGKDEEFTLKLINRPILVLRGLDGFVCHHRGSNQLDTNRSVYDVFHLSFSDGAYRIRGRDGGFWYTGSHGSVCSDGERAEDFVFEFRERGRLAIRARSGKYLRGGASGLLRADADAPAGTALWEY

SEQ ID NO: 16 - protein, 516 aa, Homo sapien
MPTNGLHQVLKIQFGLVNDTDRYLTAESFGFKVNASAPSLKRKQTWVLEPDPGQGTAVLLRSSHLGRYLSAEEDGRVACEAEQPGRDCRFLVLPQPDGRWVLRSEPHGRFFGGTEDQLSCFATAVSPAELWTVHLAIHPQAHLLSVSRRRYVHLCPREDEMAADGDKPWGVDALLTLIFRSRRYCLKSCDSRYLRSDGRLVWEPEPRACYTLEFKAGKLAFKDCDGHYLAPVGPAGTLKAGRNTRPGKDELFDLEESHPQVVLVAANHRYVSVRQGVNVSANQDDELDHETFLMQIDQETKKCTFYSSTGGYWTLVTHGGIHATATQVSANTMFEMEWRGRRVALKASNGRYVCMKKNGQLAAISDFVGPPPRPAWTGKVAGGAAQQTLSPPGKDEEFTLKLINRPILVLRGLDGFVCHHRGSNQLDTNRSVYDVFHLSFSDGAYRIRGRDGGFWYTGSHGSVCSDGERAEDFVFEFRERGRLAIRARSGKYLRGGASGLLRADADAPAGTALWEY

SEQ ID NO: 17 - protein, 492 aa, Homo sapien
MPTNGLHQVLKIQFGLVNDTDRYLTAESFGFKVNASAPSLKRKQTWVLEPDPGQGTAVLLRSSHLGRYLSAEEDGRVACEAEQPGRDCRFLVLPQPDGRWVLRSEPHGRFFGGTEDQLSCFATAVSPAELWTVHLAIYPQAHLLSVSRRRYVHLCPREDEMAADGDKPWGVDALLTLIFRSRRYCLKSCDSRYLRSDGRLVWEPEPRACYTLEFKAGKLAFKDCDGHYLAPVGPAGTLKAGRNTRPGKDELFDLEESHPQVVLVAANHRYVSVRQGVNVSANQDDELDHETFLMQIDQETKKCTFYSSTGGYWTLVTHGGIHATATQVSANTMFEMEWRGRRVALKASNGRYVCMKKNGQLAAISDFVGKDEEFTLKLINRPILVLRGLDGFVCHHRGSNQLDTNRSVYDVFHLSFSDGAYRIRGRDGGFWYTGSHGSVCSDGERAEDFVFEFRERGRLAIRARSGKYLRGGASGLLRADADAPAGTALWEY

SEQ ID NO: 18 - protein, 516 aa, Homo sapien
MPTNGLHQVLKIQFGLVNDTDRYLTAESFGFKVNASAPSLKRKQTWVLEPDPGQGTAVLLRSSHLGRYLSAEEDGRVACEAEQPGRDCRFLVLPQPDGRWVLRSEPHGRFFGGTEDQLSCFATAVSPAELWTVHLAIYPQAHLLSVSRRRYVHLCPREDEMAADGDKPWGVDALLTLIFRSRRYCLKSCDSRYLRSDGRLVWEPEPRACYTLEFKAGKLAFKDCDGHYLAPVGPAGTLKAGRNTRPGKDELFDLEESHPQVVLVAANHRYVSVRQGVNVSANQDDELDHETFLMQIDQETKKCTFYSSTGGYWTLVTHGGIHATATQVSANTMFEMEWRGRRVALKASNGRYVCMKKNGQLAAISDFVGPPPRPAWTGKVAGGAAQQTLSPPGKDEEFTLKLINRPILVLRGLDGFVCHHRGSNQLDTNRSVYDVFHLSFSDGAYRIRGRDGGFWYTGSHGSVCSDGERAEDFVFEFRERGRLAIRARSGKYLRGGASGLLRADADAPAGTALWEY

SEQ ID NO: 19 - DNA, 1684 bp, homo sapien
agaggcgggucagagcaggcaggggguucgugacgccggcugggucugggggcugugggccagccgagccgacccgggcuucugggggaccgcgggggccgugagcacucagagggcgcaucccaggccccuccggggacccggccagccugaagaugccgacgaacggccugcaccaggugcugaagauccaguuuggccucgucaacgacacugaccgcuaccugacagcugagagcuucggcuucaaggucaaugccucggcacccagccucaagaggaagcagaccugggugcuggaacccgacccaggacaaggcacggcugugcugcuccgcagcagccaccugggccgcuaccugucggcagaagaggacgggcgcguggccugugaggcagagcagccgggccgugacugccgcuuccugguccugccgcagccagaugggcgcugggugcugcgguccgagccgcacggccgcuucuucggaggcaccgaggaccagcuguccugcuucgccacagccguuuccccggccgagcuguggaccgugcaccuggccauccacccgcaggcccaccugcugagcgugagccggcggcgcuacgugcaccugugcccgcgggaggacgagauggccgcagacggagacaagcccuggggcguggacgcccuccucacccucaucuuccggagccgacgguacugccucaaguccugugacagccgcuaccugcgcagcgacggccgucuggucugggagccugagccccgugccugcuacacgcuggaguucaaggcgggcaagcuggccuucaaggacugcgacggccacuaccuggcacccguggggcccgcaggcacccucaaggccggccgaaacacgcgaccuggcaaggaugagcucuuugaucuggaggagagucacccacagguggugcugguggcugccaaccaccgcuacgucucugugcggcaaggggucaacgucucagccaaucaggaugaugaacuagaccacgagaccuuccugaugcaaauugaccaggagacaaagaagugcaccuucuauuccagcacugggggcuacuggacccuggucacccaugggggcauucacgccacagccacacaaguuucugccaacaccauguuugagauggaguggcguggccggcggguagcacucaaagccagcaacgggcgcuacgugugcaugaagaagaaugggcagcuggcggcuaucagcgauuuugucggcaaggacgaagaguucacccucaagcucaucaaccggcccauccuggugcugcgcggccuggacggcuucgucugccaccaccgcggcuccaaccagcuggacaccaaccgcuccgucuacgacgucuuccaccugagcuucagcgacggcgccuaccggauccgaggccgcgacggaggguucugguacacgggcagccacggcagcgugugcagcgacggcgaacgcgccgaggacuucgucuucgaguuccgugagcgcggccgccuggccauccgcgcccggagcggcaaguaccugcgcggcggcgccucgggccugcugcgggccgaugccgacgccccggccgggaccgcgcuuugggaguacugaggccgcgcccagaccagccugucgcgcauuaaaaccgugucucucccgca

SEQ ID NO: 20 - DNA, 1684 bp, homo sapien
agaggcgggucagagcaggcaggggguucgugacgccggcugggucugggggcugugggccagccgagccgacccgggcuucugggggaccgcgggggccgugagcacucagagggcgcaucccaggccccuccggggacccggccagccugaagaugccgacgaacggccugcaccaggugcugaagauccaguuuggccucgucaacgacacugaccgcuaccugacagcugagagcuucggcuucaaggucaaugccucggcacccagccucaagaggaagcagaccugggugcuggaacccgacccaggacaaggcacggcugugcugcuccgcagcagccaccugggccgcuaccugucggcagaagaggacgggcgcguggccugugaggcagagcagccgggccgugacugccgcuuccugguccugccgcagccagaugggcgcugggugcugcgguccgagccgcacggccgcuucuucggaggcaccgaggaccagcuguccugcuucgccacagccguuuccccggccgagcuguggaccgugcaccuggccaucuacccgcaggcccaccugcugagcgugagccggcggcgcuacgugcaccugugcccgcgggaggacgagauggccgcagacggagacaagcccuggggcguggacgcccuccucacccucaucuuccggagccgacgguacugccucaaguccugugacagccgcuaccugcgcagcgacggccgucuggucugggagccugagccccgugccugcuacacgcuggaguucaaggcgggcaagcuggccuucaaggacugcgacggccacuaccuggcacccguggggcccgcaggcacccucaaggccggccgaaacacgcgaccuggcaaggaugagcucuuugaucuggaggagagucacccacagguggugcugguggcugccaaccaccgcuacgucucugugcggcaaggggucaacgucucagccaaucaggaugaugaacuagaccacgagaccuuccugaugcaaauugaccaggagacaaagaagugcaccuucuauuccagcacugggggcuacuggacccuggucacccaugggggcauucacgccacagccacacaaguuucugccaacaccauguuugagauggaguggcguggccggcggguagcacucaaagccagcaacgggcgcuacgugugcaugaagaagaaugggcagcuggcggcuaucagcgauuuugucggcaaggacgaagaguucacccucaagcucaucaaccggcccauccuggugcugcgcggccuggacggcuucgucugccaccaccgcggcuccaaccagcuggacaccaaccgcuccgucuacgacgucuuccaccugagcuucagcgacggcgccuaccggauccgaggccgcgacggaggguucugguacacgggcagccacggcagcgugugcagcgacggcgaacgcgccgaggacuucgucuucgaguuccgugagcgcggccgccuggccauccgcgcccggagcggcaaguaccugcgcggcggcgccucgggccugcugcgggccgaugccgacgccccggccgggaccgcgcuuugggaguacugaggccgcgcccagaccagccugucgcgcauuaaaaccgugucucucccgca

SEQ ID NO: 21 - DNA, 1684 bp, homo sapien
agaggcgggtcagagcaggcagggggttcgtgacgccggctgggtctgggggctgtgggccagccgagccgacccgggcttctgggggaccgcgggggccgtgagcactcagagggcgcatcccaggcccctccggggacccggccagcctgaagatgccgacgaacggcctgcaccaggtgctgaagatccagtttggcctcgtcaacgacactgaccgctacctgacagctgagagcttcggcttcaaggtcaatgcctcggcacccagcctcaagaggaagcagacctgggtgctggaacccgacccaggacaaggcacggctgtgctgctccgcagcagccacctgggccgctacctgtcggcagaagaggacgggcgcgtggcctgtgaggcagagcagccgggccgtgactgccgcttcctggtcctgccgcagccagatgggcgctgggtgctgcggtccgagccgcacggccgcttcttcggaggcaccgaggaccagctgtcctgcttcgccacagccgtttccccggccgagctgtggaccgtgcacctggccatccacccgcaggcccacctgctgagcgtgagccggcggcgctacgtgcacctgtgcccgcgggaggacgagatggccgcagacggagacaagccctggggcgtggacgccctcctcaccctcatcttccggagccgacggtactgcctcaagtcctgtgacagccgctacctgcgcagcgacggccgtctggtctgggagcctgagccccgtgcctgctacacgctggagttcaaggcgggcaagctggccttcaaggactgcgacggccactacctggcacccgtggggcccgcaggcaccctcaaggccggccgaaacacgcgacctggcaaggatgagctctttgatctggaggagagtcacccacaggtggtgctggtggctgccaaccaccgctacgtctctgtgcggcaaggggtcaacgtctcagccaatcaggatgatgaactagaccacgagaccttcctgatgcaaattgaccaggagacaaagaagtgcaccttctattccagcactgggggctactggaccctggtcacccatgggggcattcacgccacagccacacaagtttctgccaacaccatgtttgagatggagtggcgtggccggcgggtagcactcaaagccagcaacgggcgctacgtgtgcatgaagaagaatgggcagctggcggctatcagcgattttgtcggcaaggacgaagagttcaccctcaagctcatcaaccggcccatcctggtgctgcgcggcctggacggcttcgtctgccaccaccgcggctccaaccagctggacaccaaccgctccgtctacgacgtcttccacctgagcttcagcgacggcgcctaccggatccgaggccgcgacggagggttctggtacacgggcagccacggcagcgtgtgcagcgacggcgaacgcgccgaggacttcgtcttcgagttccgtgagcgcggccgcctggccatccgcgcccggagcggcaagtacctgcgcggcggcgcctcgggcctgctgcgggccgatgccgacgccccggccgggaccgcgctttgggagtactgaggccgcgcccagaccagcctgtcgcgcattaaaaccgtgtctctcccgca

SEQ ID NO: 22 - DNA, 1684 bp, homo sapien
agaggcgggtcagagcaggcagggggttcgtgacgccggctgggtctgggggctgtgggccagccgagccgacccgggcttctgggggaccgcgggggccgtgagcactcagagggcgcatcccaggcccctccggggacccggccagcctgaagatgccgacgaacggcctgcaccaggtgctgaagatccagtttggcctcgtcaacgacactgaccgctacctgacagctgagagcttcggcttcaaggtcaatgcctcggcacccagcctcaagaggaagcagacctgggtgctggaacccgacccaggacaaggcacggctgtgctgctccgcagcagccacctgggccgctacctgtcggcagaagaggacgggcgcgtggcctgtgaggcagagcagccgggccgtgactgccgcttcctggtcctgccgcagccagatgggcgctgggtgctgcggtccgagccgcacggccgcttcttcggaggcaccgaggaccagctgtcctgcttcgccacagccgtttccccggccgagctgtggaccgtgcacctggccatctacccgcaggcccacctgctgagcgtgagccggcggcgctacgtgcacctgtgcccgcgggaggacgagatggccgcagacggagacaagccctggggcgtggacgccctcctcaccctcatcttccggagccgacggtactgcctcaagtcctgtgacagccgctacctgcgcagcgacggccgtctggtctgggagcctgagccccgtgcctgctacacgctggagttcaaggcgggcaagctggccttcaaggactgcgacggccactacctggcacccgtggggcccgcaggcaccctcaaggccggccgaaacacgcgacctggcaaggatgagctctttgatctggaggagagtcacccacaggtggtgctggtggctgccaaccaccgctacgtctctgtgcggcaaggggtcaacgtctcagccaatcaggatgatgaactagaccacgagaccttcctgatgcaaattgaccaggagacaaagaagtgcaccttctattccagcactgggggctactggaccctggtcacccatgggggcattcacgccacagccacacaagtttctgccaacaccatgtttgagatggagtggcgtggccggcgggtagcactcaaagccagcaacgggcgctacgtgtgcatgaagaagaatgggcagctggcggctatcagcgattttgtcggcaaggacgaagagttcaccctcaagctcatcaaccggcccatcctggtgctgcgcggcctggacggcttcgtctgccaccaccgcggctccaaccagctggacaccaaccgctccgtctacgacgtcttccacctgagcttcagcgacggcgcctaccggatccgaggccgcgacggagggttctggtacacgggcagccacggcagcgtgtgcagcgacggcgaacgcgccgaggacttcgtcttcgagttccgtgagcgcggccgcctggccatccgcgcccggagcggcaagtacctgcgcggcggcgcctcgggcctgctgcgggccgatgccgacgccccggccgggaccgcgctttgggagtactgaggccgcgcccagaccagcctgtcgcgcattaaaaccgtgtctctcccgca